European Patent Application EP 4 382 533 A1, published June 12, 2024. Title: Protein nanopellets for fish or teleost and crustacean vaccination. Applicant: UNIVERSITAT AUTONÒMA DE BARCELONA. The sequence listing filed with the application follows.

SEQUENCE LISTING (17 sequences)

SEQ ID NO: 1 - protein, 128 aa, Spring viremia carp virus
VEKTAGTLTTIHDNVPKCVDGTLVSGHRPGLDLIDTVFNLENVVEYTLCEGTKRKINKQEKLTSVDLSYLAPRIGGFGSVFRVRNGTLERGSTTYIRIEVEGPIVDSLNGTDPRTNASRVFWDDWELD

SEQ ID NO: 2 - protein, 149 aa, Danio rerio
SVPENLDKSIEELKAYYIKEDSQLHNAHPIFLRILKDLKVNLEESEQNLLMSIVMDTYSRIFTRMQNDSVDEATKERLAHVQEHLKKLQESYFPGKSAELRTYAETLWAIKENDPIVQRKALFELKRVYREATLLKNLKNKERKRRQAK

SEQ ID NO: 3 - protein, 7 aa, synthetic construct
GGSSRSS

SEQ ID NO: 4 - protein, 442 aa, Infectious pancreatic necrosis virus
MNTNKATATYLKSIMLPETGPASIPDDITERHILKQETSSYNLEVSESGSGVLVCFPGAPGSRIGAHYRWNANQTGLEFDQWLETSQDLKKAFNYGRLISRKYDIQSSTLPAGLYALNGTLNAATFEGSLSEVESLTYNSLMSLTTNPQDKVNNQLVTKGVTVLNLPTGFDKPYVRLEDETPQGLQSMNGAKMRCTAAIAPRRYEIDLPSQRLPPVPATGTLTTLYEGNADIVNSTTVTGDINFSLAEQPADETKFDFQLDFMGLDNDVPVVTVVSSVLATNDNYRGVSAKMTQSIPTENITKPITRVKLSYKINQQTAIGNVATLGTMGPASVSFSSGNGNVPGVLRPITLVAYEKMTPLSILTVAGVSNYELIPNPELLKNMVTRYGKYDPEGLNYAKMILSHREELDIRTVWRTEEYKERTRVFNEITDFSSDLPTSKA

SEQ ID NO: 5 - protein, 198 aa, Viral hemorrhagic septicemia virus
TVTFCGTEWIKTDLGDLIQVTGPGGTRKLTPNKCVNTDIQMRGATDDFSYLNHLITNMAQRTECLDAHSDITASGKVSSFLLSKFRPSHPGPGKAHYLLDGQIMRGDCDYEAVVSINYNRAQYKTMNNTWKSWKRVDNNTDGYDGMIFGDKLIIPDIEKYQSVYDSGMLVQRNLVEVPHLSIVFVSNTSDLSTNHIHT

SEQ ID NO: 6 - protein, 340 aa, Viral nervous necrosis virus
MVRKGDKKLAKPATTKAANPQPRRRATQRRRSGRADAPLAKASTITGFGRATNDVHISGMSRIAQAVVPAGTGTDGKIIVDSTIVPELLPRLGHAARIFQRYAVETLEFEIQPMCPANTGGGYVAGFLPNPTDNDHTFDALQATRGAVVAKWWESRTVRPQYTRTLLWTSTGKEQRLTSPGRLVLLCVGSNTDVVNVSVMCRWSVRLSVPSLETPEDTTAPITTQAPLHNDSINNGYTGFRSILLGSTQLDLAPANAVFVTDKPLPIDYSLGVGDVDRAVYWHLRKKAGDTQVPAGYFDWGLWDDFNKTFTVGAPYYSDQQPRQILLPAGTLFTRVDSEN

SEQ ID NO: 7 - protein, 156 aa, Oncorhynchus mykiss
AQFTSINMKRNIDKLKVHYKISKDQLFNGNPVFPKDTFEDSEQRVLMSVVLDVYLSIFGQMLNQTGDQEMIESLKYVKGKIQDLQKHYFLGRIPELRTHLQNLWAIETSDTTVQGKALSEFITIYEKASKLALKFHLKKDNRRKRRQAQRLKSHIM

SEQ ID NO: 8 - protein, 158 aa, Scophthalmus maximus
SHVSARMNRTIQNLLLHYKIPPKDRFNGKPVFSREPLAGKVETKKLFMVGVLETYEKLIGQMLTHLPTPNPPTTGIHVRLGAATAAATAPGAGGEVGKELNFILKKVQELRKHRYQEQSELLQGLEALGKIQMDNFVVQSKALWELPWLYEEASSISN

SEQ ID NO: 9 - DNA, 22 bp, synthetic construct
  source 1..22: mol_type = other DNA
tgtgaaggcattatggaacgaa

SEQ ID NO: 10 - DNA, 24 bp, synthetic construct
  source 1..24: mol_type = other DNA
cttccatgttgattgaaggtgaat

SEQ ID NO: 11 - DNA, 20 bp, synthetic construct
  source 1..20: mol_type = other DNA
ttatttccagaaccgggatg

SEQ ID NO: 12 - DNA, 20 bp, Danio rerio
  source 1..20: mol_type = other DNA
actcctggcattccctcttt

SEQ ID NO: 13 - protein, 134 aa, synthetic construct
VEKTAGTLTTIHDNVPKCVDGTLVSGHRPGLDLIDTVFNLENVVEYTLCEGTKRKINKQEKLTSVDLSYLAPRIGGFGSVFRVRNGTLERGSTTYIRIEVEGPIVDSLNGTDPRTNASRVFWDDWELDHHHHHH

SEQ ID NO: 14 - protein, 290 aa, synthetic construct
SVPENLDKSIEELKAYYIKEDSQLHNAHPIFLRILKDLKVNLEESEQNLLMSIVMDTYSRIFTRMQNDSVDEATKERLAHVQEHLKKLQESYFPGKSAELRTYAETLWAIKENDPIVQRKALFELKRVYREATLLKNLKNKERKRRQAKGGSSRSSVEKTAGTLTTIHDNVPKCVDGTLVSGHRPGLDLIDTVFNLENVVEYTLCEGTKRKINKQEKLTSVDLSYLAPRIGGFGSVFRVRNGTLERGSTTYIRIEVEGPIVDSLNGTDPRTNASRVFWDDWELDHHHHHH

SEQ ID NO: 15 - protein, 204 aa, synthetic construct
TVTFCGTEWIKTDLGDLIQVTGPGGTRKLTPNKCVNTDIQMRGATDDFSYLNHLITNMAQRTECLDAHSDITASGKVSSFLLSKFRPSHPGPGKAHYLLDGQIMRGDCDYEAVVSINYNRAQYKTMNNTWKSWKRVDNNTDGYDGMIFGDKLIIPDIEKYQSVYDSGMLVQRNLVEVPHLSIVFVSNTSDLSTNHIHTHHHHHH

SEQ ID NO: 16 - protein, 367 aa, synthetic construct
AQFTSINMKRNIDKLKVHYKISKDQLFNGNPVFPKDTFEDSEQRVLMSVVLDVYLSIFGQMLNQTGDQEMIESLKYVKGKIQDLQKHYFLGRIPELRTHLQNLWAIETSDTTVQGKALSEFITIYEKASKLALKFHLKKDNRRKRRQAQRLKSHIMGGSSRSSTVTFCGTEWIKTDLGDLIQVTGPGGTRKLTPNKCVNTDIQMRGATDDFSYLNHLITNMAQRTECLDAHSDITASGKVSSFLLSKFRPSHPGPGKAHYLLDGQIMRGDCDYEAVVSINYNRAQYKTMNNTWKSWKRVDNNTDGYDGMIFGDKLIIPDIEKYQSVYDSGMLVQRNLVEVPHLSIVFVSNTSDLSTNHIHTHHHHHH

SEQ ID NO: 17 - protein, 511 aa, synthetic construct
SHVSARMNRTIQNLLLHYKIPPKDRFNGKPVFSREPLAGKVETKKLFMVGVLETYEKLIGQMLTHLPTPNPPTTGIHVRLGAATAAATAPGAGGEVGKELNFILKKVQELRKHRYQEQSELLQGLEALGKIQMDNFVVQSKALWELPWLYEEASSISNGGSSRSSMVRKGDKKLAKPATTKAANPQPRRRATQRRRSGRADAPLAKASTITGFGRATNDVHISGMSRIAQAVVPAGTGTDGKIIVDSTIVPELLPRLGHAARIFQRYAVETLEFEIQPMCPANTGGGYVAGFLPNPTDNDHTFDALQATRGAVVAKWWESRTVRPQYTRTLLWTSTGKEQRLTSPGRLVLLCVGSNTDVVNVSVMCRWSVRLSVPSLETPEDTTAPITTQAPLHNDSINNGYTGFRSILLGSTQLDLAPANAVFVTDKPLPIDYSLGVGDVDRAVYWHLRKKAGDTQVPAGYFDWGLWDDFNKTFTVGAPYYSDQQPRQILLPAGTLFTRVDSENHHHHHH